European Patent Specification EP 3 475 296 B1, published April 2, 2025. Title: ARTICLES COMPRISING A SILK POLYPEPTIDE FOR ANTIGEN DELIVERY. Applicant: AMSilk GmbH, Ludwig-Maximilians-Universität München, Universität Bayreuth. The sequence listing filed with the application follows.

SEQUENCE LISTING (23 sequences)

SEQ ID NO: 1 - protein, 7 aa, artificial
  synthetic
  domain (1)..(7): Cathepsin S cleavable linker
GPMGLPG

SEQ ID NO: 2 - protein, 9 aa, artificial
  synthetic
  domain (1)..(9): Cathepsin S amd B cleavable linker
GAVGFLGIG

SEQ ID NO: 3 - protein, 35 aa, Artificial Sequence
  synthetic
  DOMAIN (1)..(35): Module C (ADF-4)
GSSAAAAAAAASGPGGYGPENQGPSGPGGYGPGGP

SEQ ID NO: 4 - protein, 35 aa, Artificial Sequence
  synthetic
  DOMAIN (1)..(35): Module Cc
GSSAAAAAAAASGPGGYGPENQGPCGPGGYGPGGP

SEQ ID NO: 5 - protein, 14 aa, artificial
  synthetic
  domain (1)..(14): T7-Tag
GCGGSGGGGSGGGG

SEQ ID NO: 6 - protein, 8 aa, Artificial Sequence
  synthetic
  DOMAIN (1)..(8): T7-Tag
GGCGGSGG

SEQ ID NO: 7 - protein, 124 aa, Artificial Sequence
  based on ADF-3
  DOMAIN (1)..(124): NR3 (ADF-3)
GAASAAVSVGGYGPQSSSAPVASAAASRLSSPAASSRVSSAVSSLVSSGPTNQAALSNTISSVVSQVSASNPGLSGCDVLVQALLEVVSALVSILGSSSIGQINYGASAQYTQMVGQSVAQALA

SEQ ID NO: 8 - protein, 109 aa, Artificial Sequence
  based on ADF-4
  DOMAIN (1)..(109): NR4 (ADF-4)
GAYGPSPSASASVAASRLSSPAASSRVSSAVSSLVSSGPTNGAAVSGALNSLVSQISASNPGLSGCDALVQALLELVSALVAILSSASIGQVNVSSVSQSTQMISQALS

SEQ ID NO: 9 - protein, 136 aa, artificial
  synthetic
  domain (1)..(136): derived from Latrodectus hesperus (NR5)
MGQANTPWSSKANADAFINSFISAASNTGSFSQDQMEDMSLIGNTLMAAMDNMGGRITPSKLQALDMAFASSVAEIAASEGGDLGVTTNAIADALTSAFYQTTGVVNSRFISEIRSLIGMFAQASANDVYASAGSG

SEQ ID NO: 10 - protein, 137 aa, artificial
  synthetic
  domain (1)..(137): derived from Latrodectus hesperus (NR6)
MGQANTPWSSKENADAFIGAFMNAASQSGAFSSDQIDDMSVISNTLMAAMDNMGGRITQSKLQALDMAFASSVAEIAVADGQNVGAATNAISDALRSAFYQTTGVVNNQFITGISSLIGMFAQVSGNEVSYSSAGSG

SEQ ID NO: 11 - protein, 8 aa, artificial
  synthetic
  domain (1)..(8): epitope of chicken-Ovalbumin
SIINFEKL

SEQ ID NO: 12 - protein, 576 aa, artificial
  synthetic
  REPEAT (1)..(576): C16
MASMTGGQQMGRGSMGSSAAAAAAAASGPGGYGPENQGPSGPGGYGPGGPGSSAAAAAAAASGPGGYGPENQGPSGPGGYGPGGPGSSAAAAAAAASGPGGYGPENQGPSGPGGYGPGGPGSSAAAAAAAASGPGGYGPENQGPSGPGGYGPGGPGSSAAAAAAAASGPGGYGPENQGPSGPGGYGPGGPGSSAAAAAAAASGPGGYGPENQGPSGPGGYGPGGPGSSAAAAAAAASGPGGYGPENQGPSGPGGYGPGGPGSSAAAAAAAASGPGGYGPENQGPSGPGGYGPGGPGSSAAAAAAAASGPGGYGPENQGPSGPGGYGPGGPGSSAAAAAAAASGPGGYGPENQGPSGPGGYGPGGPGSSAAAAAAAASGPGGYGPENQGPSGPGGYGPGGPGSSAAAAAAAASGPGGYGPENQGPSGPGGYGPGGPGSSAAAAAAAASGPGGYGPENQGPSGPGGYGPGGPGSSAAAAAAAASGPGGYGPENQGPSGPGGYGPGGPGSSAAAAAAAASGPGGYGPENQGPSGPGGYGPGGPGSSAAAAAAAASGPGGYGPENQGPSGPGGYGPGGPG

SEQ ID NO: 13 - protein, 588 aa, artificial
  synthetic
  REPEAT (1)..(585): C16-SIINFEKL
MASMTGGQQMGRGSMGSSAAAAAAAASGPGGYGPENQGPSGPGGYGPGGPGSSAAAAAAAASGPGGYGPENQGPSGPGGYGPGGPGSSAAAAAAAASGPGGYGPENQGPSGPGGYGPGGPGSSAAAAAAAASGPGGYGPENQGPSGPGGYGPGGPGSSAAAAAAAASGPGGYGPENQGPSGPGGYGPGGPGSSAAAAAAAASGPGGYGPENQGPSGPGGYGPGGPGSSAAAAAAAASGPGGYGPENQGPSGPGGYGPGGPGSSAAAAAAAASGPGGYGPENQGPSGPGGYGPGGPGSSAAAAAAAASGPGGYGPENQGPSGPGGYGPGGPGSSAAAAAAAASGPGGYGPENQGPSGPGGYGPGGPGSSAAAAAAAASGPGGYGPENQGPSGPGGYGPGGPGSSAAAAAAAASGPGGYGPENQGPSGPGGYGPGGPGSSAAAAAAAASGPGGYGPENQGPSGPGGYGPGGPGSSAAAAAAAASGPGGYGPENQGPSGPGGYGPGGPGSSAAAAAAAASGPGGYGPENQGPSGPGGYGPGGPGSSAAAAAAAASGPGGYGPENQGPSGPGGYGPGGPGGSGSIINFEKLG

SEQ ID NO: 14 - protein, 591 aa, artificial
  synthetic
  REPEAT (1)..(591): eADF4(C16-CathS-CD8)
MASMTGGQQMGRGSMGSSAAAAAAAASGPGGYGPENQGPSGPGGYGPGGPGSSAAAAAAAASGPGGYGPENQGPSGPGGYGPGGPGSSAAAAAAAASGPGGYGPENQGPSGPGGYGPGGPGSSAAAAAAAASGPGGYGPENQGPSGPGGYGPGGPGSSAAAAAAAASGPGGYGPENQGPSGPGGYGPGGPGSSAAAAAAAASGPGGYGPENQGPSGPGGYGPGGPGSSAAAAAAAASGPGGYGPENQGPSGPGGYGPGGPGSSAAAAAAAASGPGGYGPENQGPSGPGGYGPGGPGSSAAAAAAAASGPGGYGPENQGPSGPGGYGPGGPGSSAAAAAAAASGPGGYGPENQGPSGPGGYGPGGPGSSAAAAAAAASGPGGYGPENQGPSGPGGYGPGGPGSSAAAAAAAASGPGGYGPENQGPSGPGGYGPGGPGSSAAAAAAAASGPGGYGPENQGPSGPGGYGPGGPGSSAAAAAAAASGPGGYGPENQGPSGPGGYGPGGPGSSAAAAAAAASGPGGYGPENQGPSGPGGYGPGGPGSSAAAAAAAASGPGGYGPENQGPSGPGGYGPGGPGPMGLPGSIINFEKLG

SEQ ID NO: 15 - protein, 593 aa, artificial
  synthetic
  REPEAT (1)..(593): eADF4(C16-CathB-CD8)
MASMTGGQQMGRGSMGSSAAAAAAAASGPGGYGPENQGPSGPGGYGPGGPGSSAAAAAAAASGPGGYGPENQGPSGPGGYGPGGPGSSAAAAAAAASGPGGYGPENQGPSGPGGYGPGGPGSSAAAAAAAASGPGGYGPENQGPSGPGGYGPGGPGSSAAAAAAAASGPGGYGPENQGPSGPGGYGPGGPGSSAAAAAAAASGPGGYGPENQGPSGPGGYGPGGPGSSAAAAAAAASGPGGYGPENQGPSGPGGYGPGGPGSSAAAAAAAASGPGGYGPENQGPSGPGGYGPGGPGSSAAAAAAAASGPGGYGPENQGPSGPGGYGPGGPGSSAAAAAAAASGPGGYGPENQGPSGPGGYGPGGPGSSAAAAAAAASGPGGYGPENQGPSGPGGYGPGGPGSSAAAAAAAASGPGGYGPENQGPSGPGGYGPGGPGSSAAAAAAAASGPGGYGPENQGPSGPGGYGPGGPGSSAAAAAAAASGPGGYGPENQGPSGPGGYGPGGPGSSAAAAAAAASGPGGYGPENQGPSGPGGYGPGGPGSSAAAAAAAASGPGGYGPENQGPSGPGGYGPGGPGAVGFLGIGSIINFEKLG

SEQ ID NO: 16 - protein, 11 aa, artificial
  synthetic
  DOMAIN (1)..(11): sequence cleaved from the hybrid polypeptide comprising the cathepsin B cleavable linker and the epitope of chicken-Ovalbumin (OVA257-264)
IGSIINFEKLG

SEQ ID NO: 17 - protein, 12 aa, artificial
  synthetic
  DOMAIN (1)..(12): sequence cleaved from the hybrid polypeptide comprising the cathepsin S cleavable linker and the epitope of chicken-Ovalbumin (OVA257-264)
LPGSIINFEKLG

SEQ ID NO: 18 - protein, 35 aa, artificial
  synthetic
  DOMAIN (1)..(35): C kappa
GSSAAAAAAAASGPGGYGPKNQGPSGPGGYGPGGP

SEQ ID NO: 19 - protein, 11 aa, artificial
  syntetic
  DOMAIN (1)..(11): T7-Tag
MASMTGGQQMG

SEQ ID NO: 20 - protein, 5 aa, artificial
  Cathepsin S cleavage site
  domain (1)..(5)
PMGLP

SEQ ID NO: 21 - protein, 4 aa, artificial
  Cathepsin B cleavage site
  domain (1)..(4)
GFLG

SEQ ID NO: 22 - protein, 4 aa, artificial
  Cathepsin B cleavage site
  domain (1)..(4)
ALAL

SEQ ID NO: 23 - protein, 4 aa, artificial
  Cathepsin B cleavage site
  domain (1)..(4)
GGGF